European Patent Specification EP 3 167 056 B1, published September 11, 2024. Title: Milk clotting aspartic protease enzyme composition. Applicant: Chr. Hansen A/S. The sequence listing filed with the application follows.

SEQUENCE LISTING (9 sequences)

SEQ ID NO: 1 - protein, 323 aa, cow
GEVASVPLTNYLDSQYFGKIYLGTPPQEFTVLFDTGSSDFWVPSIYCKSNACKNHQRFDPRKSSTFQNLGKPLSIHYGTGSMQGILGYDTVTVSNIVDIQQTVGLSTQEPGDVFTYAEFDGILGMAYPSLASEYSIPVFDNMMNRHLVAQDLFSVYMDRNGQESMLTLGAIDPSYYTGSLHWVPVTVQQYWQFTVDSVTISGVVVACEGGCQAILDTGTSKLVGPSSDILNIQQAIGATQNQYGEFDIDCDNLSYMPTVVFEINGKMYPLTPSAYTSQDQGFCTSGFQSENHSQKWILGDVFIREYYSVFDRANNLVGLAKAI

SEQ ID NO: 2 - protein, 323 aa, Buffalo
GEVASVPLTNYLDSQYFGKIYLGTPPQEFTVLFDTGSSDFWVPSIYCKSNACKNHQRFDPRKSSTFQNLGKPLSIRYGTGSMQGILGYDTVTVSNIVDIQQTVGLSTQEPGDVFTYAEFDGILGMAYPSLASEYSIPVFDNMMNRHLVAQDLFSVYMDRNGQESMLTLGAIDPSYYTGSLHWVPVTVQQYWQFTVDSITISGVVVACEGGCQAILDTGTSKLVGPSSDILNIQQAIGATQNQYGEFDIDCDNLSYMPTVVFEINGKMYPLTPSAYTSQDQGFCTSGFQSENRSQQWILGDVFIREYYSVFDRANNLVGLAKAI

SEQ ID NO: 3 - protein, 323 aa, Goat
GEVASVPLTNYLDSQYFGKIYLGTPPQEFTVLFDTGSSDFWVPSIYCKSNACKNHQRFDPRKSSTFQNLGKPLSIRYGTGSMQGILGYDTVTVSNIVDTQQTVGLSTQEPGDVFTYAEFDGILGMAYPSLASEYSVPVFDNMMDRRLVAQDLFSVYMDRNGQGSMLTLGAIDPSYYTGSLHWVPVTLQKYWQFTVDSVTISGAVVACEGGCQAILDTGTSKLVGPSSDILNIQQAIGATQNQYGEFDIDCDSLSSMPTVVFEINGKMYPLTPYAYTSQEEGFCTSGFQGENHSHQWILGDVFIREYYSVFDRANNLVGLAKAI

SEQ ID NO: 4 - protein, 323 aa, Sheep
GEVASVPLTNYLDSQYFGKIYLGTPPQEFTVLFDTGSSDFWVPSIYCKSNACKNHQRFDPRKSSTFQNLGKPLSIRYGTGSMQGILGYDTVTVSNIVDIQQTVGLSTQEPGDVFTYAEFDGILGMAYPSLASEYSVPVFDNMMDRRLVAQDLFSVYMDRSGQGSMLTLGAIDPSYYTGSLHWVPVTLQKYWQFTVDSVTISGAVVACEGGCQAILDTGTSKLVGPSSDILNIQQAIGATQNQYGEFDIDCDSLSSMPTVVFEINGKMYPLTPYAYTSQEEGFCTSGFQGENHSHQWILGDVFIREYYSVFDRANNLVGLAKAI

SEQ ID NO: 5 - protein, 323 aa, Camel [sequence omitted]

SEQ ID NO: 6 - protein, 323 aa, Pig
GEVASEPLTNYLDTQYFGKIYIGTPPQEFTVVFDTGSSELWVPSVYCKSDACQNHHRFNPSKSSTFQNLDKPLSIQYGTGSIQGFLGYDTVMVAGIVDAHQTVGLSTQEPSDIFTYSEFDGILGLGYPELASEYTVPVFDNMMHRHLVAQDLFAVYMSRNDEGSMLTLGAIDPSYYTGSLHWVPVTMQLYWQFTVDSVTINGVVVACNGGCQAILDTGTSMLAGPSSDILNIQMAIGATESQYGEFDIDCGSLSSMPTVVFEISGRMYPLPPSAYTNQDQGFCTSGFQGDSKSQHWILGVVFIQEYYSVFDRANNRVGLAKAI

SEQ ID NO: 7 - protein, 330 aa, Cow
AATLVSEQPLQNYLDTEYFGTIGIGTPAQDFTVIFDTGSSNLWVPSIYCSSEACTNHNRFNPQDSSTYEATSETLSITYGTGSMTGILGYDTVQVGGISDTNQIFGLSETEPGSFLYYAPFDGILGLAYPSISSSGATPVFDNIWDQGLVSQDLFSVYLSSNEESGSVVIFGDIDSSYYSGSLNWVPVSVEGYWQITVDSITMNGESIACSDGCQAIVDTGTSLLAGPTTAISNIQSYIGASEDSSGEVVISCSSIDSLPDIVFTINGVQYPVPPSAYILQSNGICSSGFEGMDISTSSGDLWILGDVFIRQYFTVFDRGNNQIGLAPVA

SEQ ID NO: 8 - protein, 361 aa, Mucor
AAADGSVDTPGYYDFDLEEYAIPVSIGTPGQDFLLLFDTGSSDTWVPHKGCTKSEGCVGSRFFDPSASSTFKATNYNLNITYGTGGANGLYFEDSIAIGDITVTKQILAYVDNVRGPTAEQSPNADIFLDGLFGAAYPDNTAMEAEYGSTYNTVHVNLYKQGLISSPLFSVYMNTNSGTGEVVFGGVNNTLLGGDIAYTDVMSRYGGYYFWDAPVTGITVDGSAAVRFSRPQAFTIDTGTNFFIMPSSAASKIVKAALPDATETQQGWVVPCASYQNSKSTISIVMQKSGSSSDTIEISVPVSKMLLPVDQSNETCMFIILPDGGNQYIVGNLFLRFFVNVYDFGNNRIGFAPLASAYENE

SEQ ID NO: 9 - protein, 330 aa, Endotheia
STGSATTTPIDSLDDAYITPVQIGTPAQTLNLDFDTGSSDLWVFSSETTASEVDGQTIYTPSKSTTAKLLSGATWSISYGDGSSSSGDVYTDTVSVGGLTVTGQAVESAKKVSSSFTEDSTIDGLLGLAFSTLNTVSPTQQKTFFDNAKASLDSPVFTADLGYHAPGTYNFGFIDTTAYTGSITYTAVSTKQGFWEWTSTGYAVGSGTFKSTSIDGIADTGTTLLYLPATVVSAYWAQVSGAKSSSSVGGYVFPCSATLPSFTFGVGSARIVIPGDYIDFGPISTGSSSCFGGIQSSAGIGINIFGDVALKAAFVVFNGATTPTLGFASK